European Patent Application EP 4 563 593 A1, published June 4, 2025. Title: Increasing the photosynthesis of a plant, plant part, or plant cell. Applicant: Max-Planck-Gesellschaft zur Förderung der Wissenschaften e.V. The sequence listing filed with the application follows.

SEQUENCE LISTING (17 sequences)

SEQ ID NO: 1 - DNA, 20 bp, Cardamine hirsuta
  source 1..20: mol_type = genomic DNA; note = MRE of the C. hirsuta SPL9 gene
gtgctctctctcttctgtca

SEQ ID NO: 2 - DNA, 20 bp, synthetic construct
  source 1..20: mol_type = other DNA; note = mutated miR156 binding motif
gcgcattgagcttgttaagc

SEQ ID NO: 3 - DNA, 1851 bp, Arabidopsis thaliana
  source 1..1851: mol_type = genomic DNA; note = SPL9 gene
atggagatgggttccaactcgggtccgggtcatggtccgggtcaggcagagtcgggtggttcctccactgagtcatcctctttcagtggagggctcatgtttggccagaagatctacttcgaggacggtggtggtggatccgggtcttcttcctcaggtggtcgttcaaacagacgtgtccgtggaggcgggtcgggtcagtcgggtcagataccaaggtgccaagtggaaggttgtgggatggatctaaccaatgcaaaaggttattactcgagacaccgagtttgtggagtgcactctaaaacacctaaagtcactgtggctggtatcgaacagaggttttgtcaacagtgcagcaggttcttttattcttcttcccagttctaccctttagttctattctttattaacatgttttgccattgccggagatattcgagtccggccaaggctctgcttgttccactgttgtgaatcaaatctaaaggctttagctttttgtgattgtcagtgtcatatgcttttttggctttaacgtctttttattttcattttttaaaaaactttacagcttagttttgtaacctggtcttgtgtttgttggactcgttgggctcatttttgggaatatgtttacgtctacttgtagatgcttctcttttatttttcttttgattttgtctttctaaatatctaatccaaagagatatgaaatgaatggacaagaagaaagccgttgccctcatttttgcttctttaggtcatatcattattgagggggacaaaactagtgtaccatagcatcattgacgtgatcattgaggaactctgttacattatattacaagtgtgtggttttagattttaattcaaaactgatgacaaaagcttataatgactgatagaatgtatacaaacggtagttaacgtggagaggtcttgtctttggaatgttctgttatgttgcttttctttgaagttaactcaatctgaatcaatcacataggtttcatcagcttccggaatttgacctagagaaaaggagttgccgcaggagactcgctggtcataatgagcgacgaaggaagccacagcctgcgtctctctctgtgttagcttctcgttacgggaggatcgcaccttcgctttacggttagatccttaagctcgacacataagaccgattcatgtacttttcatccttaaaagatagatgtatatgctacagaaaatggtgatgctggaatgaatggaagctttcttgggaaccaagagataggatggccaagttcaagaacattggatacaagagtgatgaggcggccagtgtcgtcaccgtcatggcagatcaatccaatgaatgtatttagtcaaggttcagttggtggaggagggacaagcttctcatctccagagattatggacactaaactagagagctacaagggaattggcgactcaaactgtgctctctctcttctgtcaaatccacatcaaccacatgacaacaacaacaacaacaacaacaacaacaacaacaacaacaatacatggcgagcttcttcaggttttggcccgatgacggttacaatggctcaaccaccacctgcacctagccagcatcagtatctgaacccgccttgggtattcaaggacaatgataatgatatgtctcctgttttgaatttaggtcgatacaccgagccagataattgtcagataagtagtggcacggcaatgggtgagttcgagttatctgatcaccatcatcaaagtaggagacagtacatggaagatgagaacacaagggcttatgactcttcttctcaccataccaactggtctctctga

SEQ ID NO: 4 - DNA, 1842 bp, Cardamine hirsuta
  source 1..1842: mol_type = genomic DNA; note = SPL9 gene
atggagatgggttccaactctggtccgggtcttgttccgggtcaggcagagtccggtggttcatccactgagtcatcctctttcagtggaggtctcatgtttggccaaaagatctactttgaagacgctggaggtggatccggttcttcttcttctggtgggtcaaacagacgggtccgtggaggtggttcgggtcaatcgggtcagataccaaggtgccaagtggaaggttgtggagtggatctaaccaatgcaaaaggttattactcgagacatagagtttgtggaatgcactctaaaacacctaaagtcattgtctctggtatcgagcagaggttttgtcaacagtgcagcaggttcaattctaccctttagttcttatgtttatttacatgttttgccattgccggagatatatactcgagtcctgaccaaggctctatctctctttgcgtccaaactcttgtgaatcaaatcttaaagactttagctttttttgtgattgtcagtgtcatatgcttttttggctttaacgtctttttttgtttttttcaatttttttttttgaaactttacagcttagttttgtaaacctggtcttgtgtttgttggactcgttgggcttattttggggaatatgtttacgtgtacttctcttatatgcttctttaaaattttttattttggctttctaaaatatctaatcttaagagatatgaaatgaatggacaataagaaacccttagccttctttatttgcttctttaggtcatatcattattgagggggacaaaactagtgcacaccataccaccactgacgtgatcaatgaaaataaactctgttacaaatgtgtggttttttaatattcgaatttttaaaaactgatagtgacttgtaagtagaatgtatagatttagtggtttggaatgtttttagttatgttgcttttctttgaagttaactcgatctaaatcaatcaaataggtttcatcagcttccggaatttgacctagagaaaagaagttgtcgtaggagacttgctggccataatgaacgacgtaggaagccacagcctgcgtctctatctgtgttgtcttctcgttacgggaggatcgcaccgtcgctttacggttagatcctttagctctttagacctgatcactaatgtgctttaaactaaacctaagatgtgtgttttcaggaaatgctggtgatggtggaatgaacaatggaagctttcttgggaaccaagaaatgggatggacaagttcaagaacgttggatacaagagtaatgagacgacctgtgtcagcaccatcatggcaaatcaatccaatgaatgtatttagtcaaggttcagttggtggaggaggaggaggagggacaagcttttcatctccagaggctatggacactaaactagagagctacaagggaataggcgactcaaactgtgctctctctcttctgtcaaatccacatcagccacatgacaacaacaacaacaataacacatggcgaggttcttcaagttttggtcccatgacagttacaatggctcagccaccaccagtacctagtcagcatcagtatatgaactcgccttgggtattcaaggaagataataataatgatgatatgtctcctgttttgaatttgggtagattcacagagccagataattgtcagataaacaacaatgtgacaacaatggctgagtttgagttgtcagatcatcatcatcatcatcaagacaggagacagtataacatggaagatgagaacactactacaagggcttatgactcttcttctcaccataacaactggtctctctga

SEQ ID NO: 5 - DNA, 2102 bp, Brassica napus
  source 1..2102: mol_type = genomic DNA; note = SPL9 gene
atgaatatgggttccaactcgggtcagggtcttggtccgggtcaggcagactccggtggttcatcgaatgagtcatcctctttcagcggagggctcatgtttgggcagaggatctacttcgaggacggtggaggtgggtcttcttcctccggcgggtcaaacagaagggttcgtggaggcgggtcgggtcaatcaagtcagataccaaggtgccaagtggaaggttgtggagtggatctaaccaatgcaaagggttactacttgaggcacagagtttgtggaatgcactctaaaacacctagagtcattgttgctggtatcgaacagaggttttgtcaacagtgcagcaggttcttcatttcattttttttctccctattctaccccttacttcttgtgtttatttgttttgccattatccacatgcccggtcctgaacataggcaaattaatgaacaatcggtataaaacatcaccactatattatatgataattttagttgtgtatagaacattaattatataaaaaataagcaaccggcacttattgccggccaagactctcctgtgaatcaaatccaaaggctttagctatctttttgtgtagattgtcagtgtcatacgctttttcttggctttaacgtctttggagggtttcacttttaactttacagcttagtgttttgtaacttggtcttgtgtttgttggactcgttggggctcatttttgggaatatgttttacgtgtacttctatatgcttctcttttatttcttttgacttgtctctctaaaaaaaatccaatctaaagggatatgaaatgaatggacaataagaaacctattgcccttgtgtttgcttctttaggtcgtatcattattgagggggacaaaactggtaccatggcatcaatgacgtgaacactcaagaaactatgttacagacttacagtgtaacttaacaaaaaaaaactatgttacagtgtgtgtgtggttaattataagattcagaatcaagttaaccttattgacttaaagaatccattaagacgaccttatgtgtttggaacgtttttggttatatgttgcttttctagaagctaacacggtctgaatcaatgtgacatataggtttcatcagcttcaagaatttgacctagagaaaaggagttgccgtaggagactcgctggtcataatgagcgacggaggaagccacagcctgcgtctctctcggtgttgtcttctcgttatgggaggatagcaccttccctttacggttagatcattaaacctgttatgttaatcaacgaatgaaagtcctacatttggagatataataaactaatatataagtggttagagccaatctatttattatcaattaattgatttttagccaatgaaatttaacataataagcttttttcaaaaaaaaaaaattaacataataagatgacttgtaaactaaccctaagatgtatatgtttcacaatgttttggggacaggaaatgctgaaagtacaatgaatgggagctttcttggttcccaagatatgagttggacgagttcaagaacgttggatacaagagtaatgagacggccagtggcagcaccatcatggcagatcaatccaatggatgtgtttagtcaaggatcagtaagtggaggaggagggataagcttttcatctccagagattatggacactaaaccagagagctacaagggtattggcggtgactcaaactgtgctctctctcttctgtcaaatccacatcagccagcagacaacaacaacacatggagaacttcttcaggttttggtcctatgacggttacaatggctcagccaccacctgcacctagccagcatcagtatctgaacccgccttgggtgttcaaggacgatgataataactgtccgaatgatatgtctcctgttttgaacttggcccggttcaccgagacagatacgacaatgggtgagttcgagttatctgatcatcatcatcctcaacatcaaaataggaggcagtacatggaagatgataacacaagggcttatgactcttcttcacagcataacaactggtctctctga

SEQ ID NO: 6 - DNA, 1980 bp, Brassica napus
  source 1..1980: mol_type = genomic DNA; note = SPL9 gene
atggataggggttccaactcgggtcttggtcttggtccaggccagacagagtcgggtggttcatccactgagtcatcctctttaagtggagggctcatgtttggccagaggatctacttcgaggacgctggaggtggaaccgggtcttcttcctccggcgggtcaaacagaagggtacgtggaagcgggtcgggtccttcgggtcagataccaaggtgtcaagtggaaggttgtggaatggatctaaccaatgcaaagggttattacacgaggcatagagtttgtggaatgcactctaaaacaccaaaagtcattgtcgctggtatagaacaaaggttttgtcaacagtgcagcaggttctttctttttttctctcccaattctacccttaattatagtgtttatttgcatcttttgccattaccgaagtccagacgaaacattagtctataactcacaaaatatcagtgattaatatgtatatatcatttgaccccaacaatttttctaaaaaatatgtttaataaatgtttcgaaccttataaatctcagggctggctggtcggagtccggccaagaccttcctgtgaatcaaaatccaaaggctttagcttttttttttctttgtagattgtcagtgtcatatgcttttttggcttttaacggctttggaggggttctcttttaactttacagcttagtgttatgtaacttggtcttgtgtttgttgggactcgttgggcttattttggagaatatgtttacgtgtacttctatatgcttctcttttaatttttaattttaatttttattttgtctttctaaaaaatccaaagggatatgaaatgaatggacaataaagaaaacccattgccctcatatgtttgcttctttaggtcatatcattattaagggggacaaaactggtaccatagcatcaatgacatgaacactcaagaaactttgttacaatgtgtaggtcataagattcggaatcaaaatgaaaatgaaacctattagactctaaacaattcattaagaagaaatggttttacgtttttaaggattagagaggtcatttgatgtgtttggaatgtaatatatgttgcttttctttgaagttaactcgatcttaatcattaggtttcatcagcttccggaatttgacctagaaaaaaggagttgccgtaggagactcgctggtcataatgagagaaggaggaagccacagcctgcgtctctatctgtgttgtcttctcgctatgggaggatcactccttctctatacggttagatcctttatagcttgaaaacataagcagactgattcatgtgcttaaaactaaccctaaaatgcataatgttatgggaccaggaaatggtgaaacaacaatgaatgggagctttcttggttcccaagaaatgggttggaatagtgcaagaacgttggatacaagagtgatgagacggccaccgtcgtggcagatcaatcctatgaatgtgtttagtcaaggatcagtaagtggaggaggaggaggagggataagcttctcatctccagagattatggacactaaaccagagagctacaagggaattggcagcgactcaaactgtgctctctctcttctgtcaaacccacatcagccacatgacaacaacaacaacaacacatggagaacttcttcaggttttggtccgatgacggttacaatggctcagccaccacctgcacctagccagcagcatcagtatctgaacccgccttgggtattcaaggacgatgataatagctgtccgaatgatatgtctcctgttttgaatcttggtcggttcaccgagacagagataagcggtggaacgactttgggtgagttcgagttatctgatcatcatcatcaaaataggaggcagtacatggaaggtgagaacacaagggcttatgactcttcttcacaccataacaactggtctctctga

SEQ ID NO: 7 - DNA, 1954 bp, Brassica napus
  source 1..1954: mol_type = genomic DNA; note = SPL9 gene
atggataggggttccaactcgggtcttggtcttggtccaggccagacagagtcgggtggttcatccactgagtcatcctctttaagtggagggctcatgtttggccagaggatctacttcgaggacgctggaggtggaaccgggttttcttcctccggcgggtcaaacagaagggtacgtggaagcgggtcgggtccttcgggtcagataccaagatgtcaagtggaaggttgtggaatggatctaactaatgcaaagggttattacacgaggcatagagtttgtggaatgcactctaaaacaccaaaagtcattgtcgctggtatagaacaaaggttttgtcaacagtgcagcaggttctttttttttctctcccgattctacccttaattatagtgtttatttgcatcttttgccattaccgaagtccagatgaaacattcttctactataactcacaaaatatcagagattaatatgtatatatcatttgaaccccaacaatttttttaaaaaatatgtttaataaatgtttcgaaccttataaatctcagggccggctggttggagtccggccaagactttcctgtgaatcaaaatccaaaggctttagctttctttctttgtagattgtcagtgtcatatgcttttttggcttttaacgtctttggaggggttctcttttaactttacagcttagtgttatgtaacttggtcttgtgtttgttgggactcgttgggcttattttggagaatatgtttacgtgtacttctacatgcttctcttttatttttattttagattttgtctttctaagaaatccaaagggatatgaaatgaatggacaataaaaaaacctatttcccttatgtttgcttctttaggtcatatcattattgagggggacaaaactggtaccatagcattaatgacatgaacactcaagaaactttgttacaagaaactttgttacaatgtgtaggtcataagattcggaattaaattgataatgaaacctactagactttaaacaatccataaagaagaaatgttttcgtgttaaggattagagagatcattatatatgttgcttttctttgaagctaacttgatcttaatcattaggtttcaccagcttccggaatttgacctagagaaaaggagttgccgtaggagactcgctggtcataatgagagacggaggaagccacagcctgcgtctctatctgtgttgtcttctcgttatgggaggatcactccttctctttacggttagatcctcttagcttgaaaacatactaagactgactcgtgtgcttaaactaaccctaacatgggccaggaaatggtgaaactacaatgaatgggagctttcttgggtctcaagaaatgggttggaatagtgcaagaacgttggatacaagagtgatgagacggccaccgtcgtggcagatcaatcctatgaatgtgtttagtcaaggatcagtaagtggaggaggaggaggagggataaacttctcatctccggagattatggacactaaaccagagagctacaagggaattggcagcgactcaaactgtgctctctctcttctgtcaaacccacatcagccacatgacaacaacaacagcaacaacacatggagaacttcttcgggttttggtccgatgacggttacaatggctcagccaccacctgcacctagccagcagcatcagtatctgaacccgccttgggtgtttaaggacgatgataataactgtccgaatgatatgtctcctgttttgaatcttggtcggttcaccgagacagagataagcggtggaacgactttgggtgagttcgagttatctgatcatcatcatcatcagaataggacgcagtacatggaaagtgagaacacaagggcttatgactcttcttcacaccataacaactggtctctctga

SEQ ID NO: 8 - DNA, 2093 bp, Brassica napus
  source 1..2093: mol_type = genomic DNA; note = SPL9 gene
atgaatatgggttccaactcgggtcagggtcttggtcttgttcaggcagagtccggtggttcatcgaatgagtcatcctctttcagcggagggctcatgtttgggcagaagatctacttcgaggacggtgtaggtgggtcttcttcctccggcgggtcaaacagaagggttcgtggaggcgggtcgggtcaatcaagtcagataccaaggtgccaagtggaaggttgtggagtggatctaaccaatgcaaagggttactacttgaggcacagagtttgtggaatgcactctaaaacacctagagtcattgttgctggtatcgaacagaggttttgtcaacagtgcagcaggttctttatttccttctttctccctattctaccctttacttctcgtgtttattagttttgccattatccacatgcccggtcctgaacataggccaattaatgaacaatcggtataaatcatcactatattatatgataattttagttgtgtatagaacattaattatataaaaaataagcaaccggcacttattgccggccaagactctctgtgaatcaaatccaaaggctttagctatcttttttgtgtagattgtcagtgtcatatgctttttcttggctttaacgtcgttggagggtgtcacttttaactttacagcttagtgttttgtaacttggtcttgtgtttgttggactcgttggggctcaaatttgggaatatgtttacgtgtacttctatatgcttctcttttatttcttttgacttgtctctctaaaaaaaatccaatctaaagggatatgaaatgaatggacaataagaaacctattgcccttgtgtttgcttctttattgagggggacaaaactggtaccatggcatcaatgacgtgaacactcaagaaactatgttacagtgtaacttaacgaaaaaaaaaactatgttacagcgtgtgtgtggttaattataagattcagaatcaagataaccttattgacttatagaatccattaagacgaccttatgtgtttggaacgcttttggggttatatgttgctttccttagaagttaacacggactgaatcaatgtgacatataggtttcatcagcttcaagaatttgacctagagaaaaggagttgccgtaggagactcgctggtcataatgagcgacggaggaagccacagcctgcgtctctctcagtgttgtcttctcgttatgggaggatagcaccttccctttacggttagatccttaaacctgttatgtcaatcaacgaatgaaagtcctacatttggagaagtaatagactaatatataaatggttagagccaatctatttattatcaattaattgattttagccaatgaaattcaacataataagatttttttcaaaaaaaaaaatattaacataataagatgacttgtaaactaaacctaagatgtatatgtttcacaatgttttggggacaggaaatgctgaaactacaatgaatgggagctttcttggttcccaagatatgagttggacgagttcaagaacgttggatacaagagtaatgagacggccagtggcagcaccatcatggcagatcaatccaatggacgtgtttagtcaaggatcagtaagtggaggaggagggataagcttctcatctccagagattatggacactaaaccagagagctacaagggtattggcggtgaatcaaactgtgctctctctcttctgtcaaatccacatcagccacaagacgacaacaacaacaacaacacatggagaacttcttcaggttttggtcctatgacggttacaatggctcagccaccacctgcacctagccagcatcagtatctgaacccgccttgggtgttcaaggacgatgataataactgtccgaatgatatgtctcctgttttgaacttggcccggttcaccgagacagatacgacaatgggtgagttcgagttatctgatcatcatcaacatcaacatcaaaataggaggcagtacatggaagatgagaacacaagggcttatgactcttcttcacaccataataacaactggtctctctga

SEQ ID NO: 9 - DNA, 3108 bp, Arabidopsis thaliana
  source 1..3108: mol_type = genomic DNA; note = SPL9 gene promoter region
aacaaaattaaaattgtcaaccaatattaaaactttacaatagtaaatttaagatcttttcattgaaaaatgtcaaatagttatacatctccaacttaaccaataaccacagatccaaaacccaaatttgccaccatttatatatatatatatatatatacatataactaataataagaaatttagcaagtatttgatagtatttgcatcagcataaatcaaaattttctcaaaatgtctgtctagctatttcagaacctagacgtagttgtaaaactagtcaggggttaggagatcgatcaggtctttagtttcagggttaaaccaatgcagccaaacaagtggaaaccactttcactaaataaagctaaacaaaaagaacaaatcaaaacctaaacctataaaataatactatactacagtttacacagactctgatggatgatgtctatgactccgatttaacttttcatacttttcattataacgaatagatctttctttagatattgtataggtacaaattatcaaaaataaaaaaaagaagtccaaaaataaaactaatttggctttaactagcaaagagaaacaaacaaactcaaaatcaagataataattagaagaagaaaaaacccatttttgtatatttaaacatgagagaaagaggtttaacaaataaaaataagagtactgaattcatttatagggttgcttgcacatctgccgacaccaactagttcccttgaagtgtcacatcttttgttgtgttccaataactgtactgctcatatttcagtctttaatacttttaaccttttcacgatcagtataaaaaaatttcttatcatattcgtcgttactctttaactaactacagtatagaagaagaaactacctatttatagaactctgatctcctcggcagtttcctattggttaccactgctgagtatatagaatctatggagaatagtatttttaaatttagaatgttactattaacttaagtacaaatcaatatcagattatcaaaattggtatagttggatgttctatggctatggggagtctgaatattgctccctggtctcagatagatgctttcaaaatttaatactacttaaatttaaacatacatcgccacatgacccatcactatcacggttacttatggatatccaacattaaagagtaccacccaacactaggactcttataaaacacataaactccaaaattttatacctaatatccctggacaatatcaataaagttttattggtttcttttttgcaacaaacgcaagagaaatttttattcgtcacggattgaggttttacgcacaccggtacaaaagtgtctatgaagaaaataacaaaccatgcaaacgtgtttaacgggctttacaaatatgttcagaaattactcgcatgcgagattaaagaaatacaaaaaacaagtttggaaccggaggattgcaattatcatctattctatatcgcgtgtgtgtgtgtgtaaaattatgatttataatgtatcgaggtcttagattttaccttgcgatcctagagtttcgtacatatatatcgactattcaagttcttctttcatctttttgtatcttaataagttccacaaatttcgacgatagagaccatacatttgttgttatcctctactcacgaagacaaccagtctaacgttattgcataagttccacgtaaattaaaattgtgtttcttttgttaatattgaaaataggttaaaatgtcgccaaaaaataagctttgaaaacttgaggtaggaaaaaatcatggttcttttgcacatgctccggaccaatcatgtttactactaaaattcttactgcttttataataatcatctcgactggcgcgtgtagaactctagatgaatgccaagtcttattttctaattataaacgcaaataataaaaaggtttaagaatatttaaatttcacatgacaatatgacacaataaatactacttgaaaaatgatctttgaaatttcatattttctaatcaaaaacaattccttcatattttgaaatataatcgatctctcatatttaatttccaattagagaattatatccacatgatttgctttcaaatatgtctatttaacgtgtacgttgaacttgaacctatttattatttaattcattcccaaactaaaaatattttattttctaaaaaatatagtcgtaagcgtacttgtgtaaatatgttctaaagttaataatgggtttagacatttagtagaaatatatattttttggtttttggtttggttggttcggataatcaaaattttcagtattcgactaaaatacatttttgagttatatttctttacttaattttcataattgtaagtatttaaccttgtgtacgattaaaaaaaaaaaagtattttaaccttgtgtatcattcataatgtaggttttctttccattttgaaaaaaagttttgatattggttcgcattcatcagttgaaaaccaagtcaaatttatggtagattggcaatggacaaacacaaaatatcatctccatttattgccaacctcataatgccaaatggtggaccaaaaggaaaaacatgcatttatttattctcttgacataagagaaaatgcatttaacttgtcaaataattgcaaggaaaaactctataaaaagatagaaatgtgaacagtataaagtaaataaagaaatatgtgtacatgaaagacctctccaatgttcacttgctccagtttctccaagattagaaactgctacgtctctctctatagctccctcgttttgctatgtggtaattaacaacagacaacagtttttgtttgtccgtaccgttttacttactctctcactgtctttgtctattaccactctcgtctctttcttttttccttctgttctgtttctctctctaaacccaaaacagtcaaaatcagggaagccgaaattttctttgctttcttctcctttggtcctttctttaaacccgagacagttaggtttgtgtgagagagagaatgatgagtaaaaccctttctgtctgagtaagaggaaaccaac

SEQ ID NO: 10 - DNA, 3449 bp, Cardamine hirsuta
  source 1..3449: mol_type = genomic DNA; note = SPL9 gene promoter region
tttcattagtgttcacttcgattatacttgttatggagaagctcgttgagattgaaaacagttttaatcatttatttctcttgtttagactgtttagtttatgatttgaacaattattgttagaaatgtattttttgtatcttaagagacttagttagttgctcattgcccttcttatgatttggaacaaatcttaatgtctgattttttcttgttgtaaatgtttgtactttcatgtttaactgattagtttctcgtagatccgtaatgtgaaagggagtagttttacttggttgattttttgttagtctgcatgttgagaatgacatcaagattatgtttcttatgagctgtttaaagtggatcttgcaggttttgtatactgtgtttgtgttgagtgggaatttatagactatgagaagaggtagagggaaagggaagaagcagaatgcatctgctcgggaagaagaagaaaagattccatcttacaggagaagaggaaggccacagaagccaatgaaagatgatttcgaagaggaagaagaagaagaggaagaggaagagatggtagagaagatagaagaagaagaagttgatgatgatgatgatagaataataagtaaagatttgaagaacgagaagaagaggaagatacctaatggaagtaatacagatgagaatgggttaggatcgaaatcaagcaccgatgattccactaagtcgatatctattgggtttagacaaaatggaagccggaggaaaagcaagccgagacgagctgctgaagctgttgtggaatgtaatggagtttgagaaatcttgtgatgaaacaaacaacttcaagatacagggtgacaaattaacctaaggcttcttcttcttactttttttttttttgttgttgcttttcttacaagtcttttgaagttgacaactttggatctttctttttagtgtttaaattatttcatgaatcaacaacatcaacctgcatacacttttctttcttgtcttttattcatctgtttggtttctctgagatttgagggtccaaagatggtcctgtaagaaatgaatttggtaatagaggttgggagagaaagtggttgacactttttgagatagatgtgagatcctctcatctcctaaagtttacattctagagatgttataattgcaaatcttgcaggttaagcatattataacaacagagcagttaagggaagagagctgagagttttggtatttttttttctttctttttgtcagcaataagggaatagtaaacaattttaacccaaaaaatagacaaagaaagaagaagagatttttcaagtatagcataaatcatatttttatgagtgtctagctatatagaacctagttggttttgtgacaacatatttgtattgtaaaatcacttttagatcaggtctttagtttcggggtttaaccaatgcagccagacacatggaaactactttcactaaataaagctaagcaaaaagaacaaatcaaacctaaacctattaaaagatgaagtgttacagttttacacagactctgatggatgtctatgacaaagatttaacttttcataccttttttattttaacgaaaatcaagaaagatcttactttggatattgtgagactcaaaattaatcaaaaaaggaagaataccaaaattaaactaatttaaggctttaatttgaagaaaaaaaatcaaacaaaccaaaagccaaaatattagtactaaaagacatttcgttatacaattcactaataaacaagagaaattaagaggtttaacaaataaaaataggtactgaatttatttatagggttgcttgcacatctgccgacaccaactagttcccttgaagtgtcacatcttttgttgtgttccaataaatgtactgttcatatttcagtcttttaatattttaagatttacaatcattatagttctaaattcactattttttttctatcatactcgttgctctttaactactacagtgtagaaaccctctatttttagaactctgaactcttcgtcagtttccttttggttcccaattctgagtatagaatctatcaaggataaaatttaagattaaaaaggttattattttaagaaacaaaaaaatatcagattatgaagatgtgtaaagttggatgtcttattcgatcagtctgaagattgctccctggtgtcaaatagatactcttaaaatttaatattcaatagtactattttaatttaaacttacatcatctatgccccataagaacttacatcacacatgacccatcaccatcacatgattcacatttaattatggatgtccaacattggaataccatggaacgtaggactcttattacaaacacatggaatccaaaaaaaattacgctacaatccatggacaagagaaataaatcttaaggttttgtctagatttttaaactttatacattgtaattattacaagtaacaaaaatttccaaagaaataacttcttgaaaagttttcttttgtttttcggtaaatatcttgaaactaacactaatagaatccatttattattaacttggtgatgatatattcgagctaaacaaaattggtgtagaggtcttcttctcctaatttccaacacacattttcaaatatgtgaagcaacagctgattatgatgctataaaaaaaacagctggttatgaaagtttaaacaagtaaaacttattttattttagctagttttaataaaattcactttcagattcatagcctaagttagattcggtttgaaaacagttggatatgagttcactaaataccaagtaaaatttatagtagatttggtatgggcaaacacaaaatatcatcttcatttattgccaacctcataatgccaatggtggaccaaaaggaaaaaacatgcatttatttattcttttgacataagaaaaaaaatgcattaacttgtcaaataattgcaaggagaaaaaaatctataaaaaggtagaaaatgtaaacagtataaagtaaaaaaagacttgtgtacatgaaagatctctccaatgttcacttgctccaagtttctctaagattagaaactgctacaactctctctttttctcttgtttttttatttgctttgcggtaatcaacagacaaccgttttttttttcttttcttttcttgtccgtaccgtttttacttactaggtctcactgtctttgtctattaccactctcgtctcatttttcttctgttgtgtgttctctctttctttctctaaacccacaacagtcaaaatcagggaagccaaaattttctttgctttcttctcctttggtcctttctttaaacccaagaaagttaggttagagatagaatgatgagtaaaaaaaacctttctgtctgaagaggaggaaaccaaaa

SEQ ID NO: 11 - DNA, 3289 bp, Brassica napus
  source 1..3289: mol_type = genomic DNA; note = SPL9 gene promoter region
gttcatctcgtctacaaaagttataattagtctaagatattataattgcaaatcgtgtacgttaggtaaaatgtagcagtaaagccattaaggaagagagttaagaaaaagggcagagtcattacactttttcttgaagtcattacacttaagagacaggtctacacaattttttttaaaaaaaattataatatatattcataatctaaaagtctaaaacaacttaagaaacttacagaaaaaagccttgaattgtttagaaaaaaatgttaattatttttaaaacatatggttaatcatttgaattatgtgagaaaaaaaaaactaaacatatatactaatgttttagtatattttagtatctctgtctaactaatgatcaacccacactccaaatggtagtgacttgaagccaagagcacttttaatgaagtttcttctcattggaatttttaatatatgtgttatatatatataaataattgtgggatccataatttttgtagaacttcataaaaatggtctaaggttacttaagaccaaatggatcgtataggaaattcaaaccctagttcccatcttttcttcaacaaatagaaaaaaagttgaggagttttttttgttttgaacaaaaaaaaagagttgaggagtttatgacattttttaagtattacatcatattcaactataatgacgacataataatattttttctgaatgtatagctatccagaacctagttgtttctgtgtgtgacacatgtttgtaaaatcagtcttgagagatcaggtctttagtttcagggtttaaccaatgcagccaaacaaaaggaaactactttcactaaataaagctaagcaaaaagaacaaatcaaacctaaacctatatattatataatatgtaaagtattacagttcgcacagactctgatggatgtctattacttttcatactttctattattacaaaaaccaggaagatcttgctttggatattgagttgtgaagttgtgaccataattttccaaacaaatcaaatggggagaaaaaaccaaatactaaaattttatttacaaaacaacaagcaaacaaagtgaaatccaaaataattaaaaacattttttggttatagcttaatatatttattgtgttgcttgcacacctgccgacaccagctagtttccttgaagtgtcacatcttttgttgtgttccaataaatgtactgctcatatttcagtcgttaaaattttaactttttaacctttaaaatcactataattaaaaattcacaatcatttttttaccatattcgttactttctaactactacagttacatttgtaaaagtaagaaacactctatttatagaactctgaactcctcggcacttgctttgtggttcccaatgctgagtatagaatctatgaaggataacagcatttgaagaccaaaatgtcattagtttaagtacaaaagaatcagattatcaagatttgtgaagttgggtgttctatgcaagtctcaagattgctcccttgtctcagataagatgctctcaacaaattcaacacagattttaattaagcttacatctcctatgacccaaaaaaaaacgtacatcacacatgacacatcaccataaactgattacatcacctatgacccaaaagaacttacatcaccacatgacacatcaccatctcatttaattatggatgtccactttaaggagaaccatcgaactagaactcctattgtaacacatcgaatccatataatgtagacacacaagaaagttatagtggaccatataggtttttaaagttaataattgatgctttttagatgcgaacggcctgataataaaactgtaggtgagaacgatttatgtgagctagatactgtatatagcgctgaatcaataaacttatgcgtatgagagaatgataacacacatttgtcaagaagaaaaaagtatgctcttagcaaaaaataaaaaaaaaagaagaaaaagtatgcatagcgagagaaaatatgggtctaaaagatgctagcatggggcaagcggtgaatatgatgagtacttgatattgtattgtgttgaaaaaacgtaaatggtcgagcttgtctagtagtatggtatacaatgaatacttaaaggccgcaacctaggtttgacgttcatatgagtgtgtttcgctcattataacgtgaagtcaatacatcccatattcacgctgagctgatcttaaacttttttttacaccgatcattcaagttcttatccgatattctgtaactgaataagtttttacatttttctactgttgatcatttacatactcacatctaaagaataaggttttaagctatataaaacttaaaccgatctcataattaacctccttacatctattttctaacagcttacttttagtgtatattcaaatgattttctttcaaacatgcatgcttaacgtgtcaaaatcaattccaaaacaaaaataaagatttcatttccttaaaaatatgtggccgcaagcaagcgaatcaagtaactactatctaaaaacggaatatataacgggattagttgaaagatattttggtttggtttggttggttggttgggataattttcaccacagttggttgataagcatttagtttgagtactctatttaattctattccgtttattttggtttgataaacattcagctcagaacttagttcaaaacccagtcaaatttgtggtagattttggtgttcagaaacccaaaatatcatctccatttattatttgccaacctcataatgccaatggtggaccaaaagaaaaacatgcatttatttattcgtttgaaaaaaaaaaaagagagaaacaaatgcgtttaacttgtcaaataattgaaccgaaaaaaatctataaaaaagttgaaaacgtgaacagtataaagtaaaaataataataaaaagatgtgtacatgatgaaagacctctccaatgttcatttgcctcaagtttcttctaactccaagattggaaactgctacatctctctctaacagacaacagtttagtctgtgtccgtaccgttttacttactgtctttgtctatcgccactctcgtctctttttctttgcttctattgtctccctctctctctctcttgtttgctttcttcccctttcgtcctttctttaaaccaagacagttaggtttgagagagagagagagaatgataagcaagtactctctttctgtctgaataaaaggaaacaaat

SEQ ID NO: 12 - DNA, 3000 bp, Brassica napus
  source 1..3000: mol_type = genomic DNA; note = SPL9 gene promoter region
ttgctggaagttggagaccctcagagagttattttttgaggaggatgttaacagaatcatcaagatgaagattgtggccaatcaagatgacttctgggtatgggttcataacaagaatggcagttactcggtgaaatcggggtattggttcattaataggctgaggaaaagcgaattagttagagaggctgaggcaagaccttccctaaatgatcttaagggagcggtgtggaagatcaaaacggctccaaagattaaaactttcttctggaaggctttgagcaatgcaattccggctggtgagttgctggtaatgaagggcgtcagattggatccgtgttgtcaagcctgtggtttcaatggtgaatctattaaccatatcttgtttgaatgctccatcgctagacagatttgggccttagcaaatgtgccatcacctatcaacggtttcgataaggtctctcacttctccaacttgcattatgttatgagtctgttatccaacaagaatgtggctgaggaaacaaggaatatgatcccttggatagtgtggtatttatggaaaactagaaatgggatcatctttgaaggaaaagcttttgtggcacatgatgtggtgagtaaaatctcagaggaagcggaattttggtgcatggcacagaagctggagaaagagaaagaagaggaggagagaaagagcagagagatggtgcagaagcgttgggaaaggccctgtgcaggatggttaaagtgcaacattggggttgatttcaacaagcaaaattcaaaaagtggaggagcttgggtggtgagaaacgagaagggcaaagtgttgttacatagtcgccgagttttttccaacattgattccctggatgaagctaaatttcaaggtctgctatggacccttgacagtctctgttctcatcgtcttaacagggttatgattgcaatcgatgatgacactttgacgaaagtaattttaaggccaaaggcatggccaagcttcagagctcaatatatggagattgagagaagactgagaagaatggaatggtggaggatagtgaaagaagaaagatcaactaacagaggggctttcctcatagctcagagtgcagcaagaggtggtttcatccaatcgtatgtggcaactggtggcccttcttggctgagacagctctttgagaatgaggaagtttctccctgtgattagctgacatgggtcaggcttttggtggctattttttggtacacgcgtttggaattttttgttgttggcttgtagtatgaagctttggctgtttgtttagcttctctgctctattgtattatgagtaggttttaaagtcggggttatgatctttgtagaagaacgttgatgtggttaaccgttttttaatataatagatgacaaaaaaaaaaataagtacagaaaatcagtattaagatctgtaaagttggatgttctatgcgagtctgaggattagatgctccctggactcagatagatgctcccaacaatttaatattactttaaatttgaacttacatcacctatgacccatgaaaaattacatcacacatgacccatcaccatcgcatttaataatggatatccaacattagggagaaccaccgaaccagaacaactctcattataaaacacaacaagaatacaaccaaatagtttagttttttttttttttcaacacaaccaaatagtttagttttatctggtaattaccacttctaagatgcgagcagcctgataataaaactgtagatgagaacaatttgtgtaagccagatattgtagatatcacggaccaacaaacttgagaagcgtacgagagaatgatatcactcatttttcaatatgagaagtatgcataacgagagaaaatatgggtctaaagaagcatgaaccaagcgatgagtacttgttgttgtgtgctgtgttttcactcattacgtgaagtcaatattctcaaagtctatgctacgatattagattgtttgtacatcaaccatgcaagttcttttccaatatttttattgatgatttatataatcttggctgagcactgattaattgattgttttcaacctattgattaacagcttaagtttagtatattttcaaaacataacatgcatatgtaacgtgtcaacctaaaaatatgtagtcacaagcgtatcatgcaactatgatctaaaaaggagtaacagggttagatggatacttagtttggttggttcgaatagtttttcattatttacttattacgttaacaaaccatatacttttgagtaatatatttagtggaaaattttattttggtttcatatctgtttgcattcaactcggttcaaaaccaagtcaaatatgtggtagattttgcaaatggagaaacacaaaagaccatctccatttatttttgccaacctcataatgccaaatggtggaccaaacgaaaaacatgcattattaattttcttggcataagaaaaaagaaatgtgttagcttgtcaaataattgaaaggagaaaaaaatctactaaaaggttgaaaatgtgaacagtataaagtaaaataattaaaatgtgtacatgaaagaaagacctctccaatgttcatttgttcaagtctcttccaactccaagattagaaactgctactacatcactctctatctctcgtttttgttatgtggtaattaacagacaacagtttatgttttgtccgtaccgttttacttaactctctcactgtctttgtctattaccactctcgtctcttttcttgcttctgttgtgtctctctctatcttctttctttaaacccaacaacagtcaaaatcagggaagccaaaattttctttgctttcttctcctttcgtccttgcctttaaaccgagacagttaggttttaagagagagagagagagagaatgatgagtgagtactccctttctgtctgagtaagaggaaacgaaa

SEQ ID NO: 13 - DNA, 3082 bp, Brassica napus
  source 1..3082: mol_type = genomic DNA; note = SPL9 gene promoter region
gttaaatttattcatgcaaaaaatgcagctatttatgaatcaaagaatcagactcatgaaactaagagacaaaatttctatgtttaataatcctctctagaaccaaaccatatagcaagctctccttccattttcctccttctttagagtgaaagcaaccaaagcctaacagttttctccacaaactttgttagacactgagcttctctttcttgttcaccatgtcgtcgagcattgcactctctccgtattgagtgaacaaccgcttggaaaacatatcggacaaggaagttttttatgggagtaagcccaggcctggtgatgatcgcaatgagctgactctagtctgtgatgaatctgttttgcaacaaaccctctgctagagccttccaggcctatcttgtgtacctgcagctgaagaatagatgttcacatgtttcttaagcttcgttacacagagtgcaggtcgcatttatcccagtgttccataaccgcattttatctcctgtttgcagtctgttgagcacagcgatccaaacaagggtggagaactttggagtcgaatgggtaaaccagatgcctctgctccagttgcaagtttggtggcagtggtgaatctgttcccaggttcttttagcagaaaatctgctgacaaatctaccttcctcttgcttccatagagcaatgtcatcaccctggttcgcagccaaacgaagagtctatttcattctccacctcatttaaaatgctcactttgtgtcttctccttcttcgttgtctaacaagaacatctgataccaaggcattatcaacaatgcctaaatcaatcagaccgcgatcacccagagcaactttaaggcagccatgcttggaccagacatcataccagaaggaagtatgcttcccattccctacttccatatggagaaactgtgttgcaagttctcggtgcttgagaagtttcctccaaacccatgagccagaggttgtagtactgctaactgaccagaaggatcccttcttgaagagatagcagtgaatccatcggacccataacgaagatttttcagaagagattcgccatattagcttcaagcagaagactgtgttcatttccttcagcggtcttaatcccgaatctccctcattctttggtaaacacagatccttccaacagacttttgcttttgatgatttgagctcaggtcccgaccaaagaaaggcagaacaaaggctctcgatctccttcagacaactgcttggtaaggtgaaagcttgcatccagaagttggtcatgctggtaatgacagagttgatgagttgcaatttgccagcgtgggagagaaatcttcatgtccaagacttcattcgtttcctgatcttctcaaccagaggcatgtagtcggtgatcatcatacgctttgtgagcaggggaagtcccaagtagcggactggtagtcgaccagatgccagagggaagctgccgaggatatttgtctctgtgtctgctgaagtaccagcaatgtatagcgttgacttctccagactgatgtttaatttcgatatagcggcaaactcttcaaaaactttgagcactctttctatagaacgtttggttccatcagtgaacaccatcagatcatcagcgaaacacaaatgtgttacctgaatattcttacacttaggatgatagccaaccagattcctctccactgccttgtcaagcatgctaggtaagacgttgatgagtacttcttgttgtgtgcggtgttgaaaaatagaacttaaattgttgtgctttgtctaggacgcaagtacttaaaggtcgtaacctaggtgtgacgttcacacgtatgttttcactcattgcgtgaagtcaatattctcaaagtctatgctacgatattagattgttgtacatcaaccatgcaagttcttttcccatatttttattgatgatttatataatcatggcactgagcactgattaattgattgttttcaacctattgattaacagcttaagtttagtatattttcaaaacataacatgcacatgtaacgtgtcaacctaaaatatgtagtcacaagcgtatcatgcaattctatgatctaaaaaggggtaacggggttagatggatacttagtttggtttttagtttggttggttcgaatagtttttcgttatttacttattaggttaacaaaccatatacttttgagtaatatatttagtggaaatttttattttggtttcatatatatatgtttgcattcaactcggttcaaaaccaagtcaaatatgtggtagattttgcaaatggagaaacacaaaagacgatctccatttattgttgccaacctcataatgccaaatggtggaccaaacgaaaaacatgcattattaattttcttgacataagaaaaaggaaatgtgttagcttgtcaaataattgaaaggagaaaaaatctactaaaaggttgaaaatgtgaacagtataaagtaaaataattaaattttaaaagatgtgtacatgaaagacctctccaatgttcatttgttcaagtctcatccaactccaagattagaaactgctactacatcactctctatctctcgtttttgttatgtggtaattaacatacaacagtttttgttttgtccgtaccgttttacttaactctctcactgtctttgtctattaccactctcgtctcttttttttcttctgttgtgtcttccaactccaagattagaactagctactacatcactctctatctctcgttttgttatgtggtaattaacatactaacagttttgttttgtccgtaccgttttacttaactctctcactgtctttgtctattaccactctcgtctcttttttttcttctgttgtgtctctctatcttctttctttaaacccaacaacagtcaaaatcagggaagccaaaattttctttgctttcttctcctttcgtccttgcctttaaaccgagacagttaggttttaagagagagagagagagagaatgatgagtgagtactccctttctgtctgagtaagaggaaacgaaa

SEQ ID NO: 14 - DNA, 3281 bp, Brassica napus
  source 1..3281: mol_type = genomic DNA; note = SPL9 gene promoter region
gactttcttcttactgcgatttggtcctttagcttttgattaatcatgatttttgccctaaacatttacagatacacatattttttctctgattttggctcaaacattttaatcatgataattaaattctgctatctttttacatttattctgtcaattcatacacactttttttgttttgttttatctttataggaagaattcatttaggtggacaatatgtaaggaagaaaggctgaacacccttttgtacatgtggatgtgtaaaccgatgtacaaccaggtcgcacacacccttttgtacatgtggatatgtataatgatatacacatatatatcactaaaacattgtacatgttgaaatttcaaatgagatttgtacttttactagctgactgaacccaaatatcatccttcacaccttgtttaagagcttctgataattagtgtgtgtatttcatgctagcttcatggtaggtcttagcttgattaatttatggttgttttacatatgtacactatcatattctcgtacacatgtacaccaccatattttatgtacacatgtaagctattatactttatcgtacactattataatttatggttgttctcttttaatttgtgtctgtctggaaaatttgtttacatattgaagaacatacattacatgggtttgtttagtaaagttggaaacatatttaggcagcctagagcgatgtagccataaacgctcgtttcattgagtttttgggttccgggtataagtttctactgatttaggatcagtgaaaacatcgaataattactgtgtttttgttgttgagtccgacctaatacattggtccttattgtttcttcaacttgagtttatcgcttttgtaagcttggtatcgatgaacttcttgctgatatatgaaaagtcttgggcttaaagtcctacatctttttgtttcaccaggtatgagaaaaattaaatgcatcggaatgtagtcacacatgtttctgtctcagcagctgatgttgtgtctacaagatgtacatccatttccgataagagcatgttactaataaagtgtacacgctgatgtttgaaaatcggtgtacatgtggatttttgtaactcattgtacatgtggataataaaaattaagtgtacacgtgcatgtacccacaaactctagtataatgtttacaactcaaccctcggacatgcatacacaccaacttttgtacaagtgtacacgtggacatgtaaaccaggatcgcatgttaaacatgtgctagattaagaacaaataaatggcatggaaggggatgatgcagaggaatggaagaatcccgagagattcggttaagtcatcgttcaccaccggaggattaaggaaaccgatagcggagataagcgttgtgaggagcagctgagccaatatatattatagatcttgcggatgaaaccccatcagaattaattctcgccgtagcttagccatgtgtaaagcgccgccgcaccaactcccatcttcaaatcaatatccttcccggcggagcaatctagccagctcatgcccacgcttgcgtatccgtagggtttcttcatggctcaacaaattgttttcgcaacagaactgaggaaatatgcttcctctgtgacgtcatcttcagcctacagtctccgtcgtcatacaaatcttaaactccggcgtgatgttctcaaatttattcaccatacttcttacatagcttagagtgaaaaagataagaaaaaaaatattaaacatgtggctgaaaataaaaagcaatgtactgtttttgttattttaaaaatttaaaataaaaaaattgaccagcaaataaaaaaccggaagctattatagttaatgtttagttagaggcatccaggtaaacaaccaataaaaactattttggtagctggaactgtcttatgttgtaataaaaacatgaaaactgctctgcagttaataactcaagaaaaagtatgcataaggagagaaaatatgggtcgaaaagaagctagcatggggcaagcggtgaataggatgagtactttgttattgtattgcgttgaaaaaaacctaaattgtcgagcttgtctactagtatgatggtatacaatgtagtatgatggtatacaatgaatacttaaaggccgcaacctaggtttgacgttcatatgagtgtgtttcgctcattataacgtgaagtcaatacatcccatattcatgctgagatgatcttaaactttttttacaccgatcatacaagttcttatccgatattttgtaactgaataagtttttacattttctactgttgatcatttacatactcacttctaaagaataaggttttaagctatataaaaacttaaaccgatctcataattaacctccttaaatctattttctaacagcttacttttagtgtatattcaaatgattttctttcaaacatgcatacctaacgtgtcaaaatcaattccaaaacaaaaataaagatttcatttcctaaaaaatatgtggccgcgagcaagcgaatcatgtaactactatctaaaaacggaatatataacggggttagttgaaagatattttggtttggtttggttggttgggataattttcactacaattggttgataaaaatttattttgagtactctatttaatactattccgttgattttggtttgataaacgttcagctcagatcttagttcaaaaccaagtcaaatttgtggtaggttttggtgttcagaaacccaaaatatcatctccgtttattatttgccaacctcataatgccaatggtggaccaaaagaaaaacatgcatttatttattcatttgaaataaaaaagagaaagaaatgcgtttaacttgtcaaataattgaaccgaaaaaaatctataaaaaagttgaaaacgtgaacagtataaagtaaaaataataataaaaagatctgtacatgatgaaagacctctccaatgttcatttgcctcaagtttcttctaactccaagattggaaactgctacatctctctctaacaaacaacagtctagtctttgtccgtaccattttacttactgtctttgtctatcgccactctcgtctcttttttatgcttctattgtctctctctctcttgtgtactttcttcccctttcgtcgtttcttcaaaccaagacagttaggtttgagagagagagagagaatgataagcaagtactctctttctgtctgaataaaaggaaacaaat

SEQ ID NO: 15 - DNA, 5974 bp, synthetic construct
  source 1..5974: mol_type = other DNA; note = rSPL9 construct
ctggcgaaagggggatgtgctgcaaggcgattaagttgggtaacgccagggttttcccagtcacgacgttgtaaaacgacggccagtgccaagctggccgctctagaactagtggatctcgagatttctaatgagtgtgaagatgctataattgcaaattgtggaacttaggcaaaatataaaacagcaaagcccttaaagggaagagaactaagaagtgagaaaggagtaattagactttagagattagtctaaattgaaaagttaaaacaaaattaaaattgtcaaccaatattaaaactttacaatagtaaatttaagatcttttcattgaaaaatgtcaaatagttatacatctccaacttaaccaataaccacagatccaaaacccaaatttgccaccatttatatatatatatatatatatacatataactaataataagaaatttagcaagtatttgatagtatttgcatcagcataaatcaaaattttctcaaaatgtctgtctagctatttcagaacctagacgtagttgtaaaactagtcaggggttaggagatcgatcaggtctttagtttcagggttaaaccaatgcagccaaacaagtggaaaccactttcactaaataaagctaaacaaaaagaacaaatcaaaacctaaacctataaaataatactatactacagtttacacagactctgatggatgatgtctatgactccgatttaacttttcatacttttcattataacgaatagatctttctttagatattgtataggtacaaattatcaaaaataaaaaaaagaagtccaaaaataaaactaatttggctttaactagcaaagagaaacaaacaaactcaaaatcaagataataattagaagaagaaaaaacccatttttgtatatttaaacatgagagaaagaggtttaacaaataaaaataagagtactgaattcatttatagggttgcttgcacatctgccgacaccaactagttcccttgaagtgtcacatcttttgttgtgttccaataactgtactgctcatatttcagtctttaatacttttaaccttttcacgatcagtataaaaaaatttcttatcatattcgtcgttactctttaactaactacagtatagaagaagaaactacctatttatagaactctgatctcctcggcagtttcctattggttaccactgctgagtatatagaatctatggagaatagtatttttaaatttagaatgttactattaacttaagtacaaatcaatatcagattatcaaaattggtatagttggatgttctatggctatggggagtctgaatattgctccctggtctcagatagatgctttcaaaatttaatactacttaaatttaaacatacatcgccacatgacccatcactatcacggttacttatggatatccaacattaaagagtaccacccaacactaggactcttataaaacacataaactccaaaattttatacctaatatccctggacaatatcaataaagttttattggtttcttttttgcaacaaacgcaagagaaatttttattcgtcacggattgaggttttacgcacaccggtacaaaagtgtctatgaagaaaataacaaaccatgcaaacgtgtttaacgggctttacaaatatgttcagaaattactcgcatgcgagattaaagaaatacaaaaaacaagtttggaaccggaggattgcaattatcatctattctatatcgcgtgtgtgtgtgtgtaaaattatgatttataatgtatcgaggtcttagattttaccttgcgatcctagagtttcgtacatatatatcgactattcaagttcttctttcatctttttgtatcttaataagttccacaaatttcgacgatagagaccatacatttgttgttatcctctactcacgaagacaaccagtctaacgttattgcataagttccacgtaaattaaaattgtgtttcttttgttaatattgaaaataggttaaaatgtcgccaaaaaataagctttgaaaacttgaggtaggaaaaaatcatggttcttttgcacatgctccggaccaatcatgtttactactaaaattcttactgcttttataataatcatctcgactggcgcgtgtagaactctagatgaatgccaagtcttattttctaattataaacgcaaataataaaaaggtttaagaatatttaaatttcacatgacaatatgacacaataaatactacttgaaaaatgatctttgaaatttcatattttctaatcaaaaacaattccttcatattttgaaatataatcgatctctcatatttaatttccaattagagaattatatccacatgatttgctttcaaatatgtctatttaacgtgtacgttgaacttgaacctatttattatttaattcattcccaaactaaaaatattttattttctaaaaaatatagtcgtaagcgtacttgtgtaaatatgttctaaagttaataatgggtttagacatttagtagaaatatatattttttggtttttggtttggttggttcggataatcaaaattttcagtattcgactaaaatacatttttgagttatatttctttacttaattttcataattgtaagtatttaaccttgtgtacgattaaaaaaaaaaaagtattttaaccttgtgtatcattcataatgtaggttttctttccattttgaaaaaaagttttgatattggttcgcattcatcagttgaaaaccaagtcaaatttatggtagattggcaatggacaaacacaaaatatcatctccatttattgccaacctcataatgccaaatggtggaccaaaaggaaaaacatgcatttatttattctcttgacataagagaaaatgcatttaacttgtcaaataattgcaaggaaaaactctataaaaagatagaaatgtgaacagtataaagtaaataaagaaatatgtgtacatgaaagacctctccaatgttcacttgctccagtttctccaagattagaaactgctacgtctctctctatagctccctcgttttgctatgtggtaattaacaacagacaacagtttttgtttgtccgtaccgttttacttactctctcactgtctttgtctattaccactctcgtctctttcttttttccttctgttctgtttctctctctaaacccaaaacagtcaaaatcagggaagccgaaattttctttgctttcttctcctttggtcctttctttaaacccgagacagttaggtttgtgtgagagagagaatgatgagtaaaaccctttctgtctgagtaagaggaaaccaacggtaccatggagatgggttccaactcgggtccgggtcatggtccgggtcaggcagagtcgggtggttcctccactgagtcatcctctttcagtggagggctcatgtttggccagaagatctacttcgaggacggtggtggtggatccgggtcttcttcctcaggtggtcgttcaaacagacgtgtccgtggaggcgggtcgggtcagtcgggtcagataccaaggtgccaagtggaaggttgtgggatggatctaaccaatgcaaaaggttattactcgagacaccgagtttgtggagtgcactctaaaacacctaaagtcactgtggctggtatcgaacagaggttttgtcaacagtgcagcaggttcttttattcttcttcccagttctaccctttagttctattctttattaacatgttttgccattgccggagatattcgagtccggccaaggctctgcttgttccactgttgtgaatcaaatctaaaggctttagctttttgtgattgtcagtgtcatatgcttttttggctttaacgtctttttattttcattttttaaaaaactttacagcttagttttgtaacctggtcttgtgtttgttggactcgttgggctcatttttgggaatatgtttacgtctacttgtagatgcttctcttttatttttcttttgattttgtctttctaaatatctaatccaaagagatatgaaatgaatggacaagaagaaagccgttgccctcatttttgcttctttaggtcatatcattattgagggggacaaaactagtgtaccatagcatcattgacgtgatcattgaggaactctgttacattatattacaagtgtgtggttttagattttaattcaaaactgatgacaaaagcttataatgactgatagaatgtatacaaacggtagttaacgtggagaggtcttgtctttggaatgttctgttatgttgcttttctttgaagttaactcaatctgaatcaatcacataggtttcatcagcttccggaatttgacctagagaaaaggagttgccgcaggagactcgctggtcataatgagcgacgaaggaagccacagcctgcgtctctctctgtgttagcttctcgttacgggaggatcgcaccttcgctttacggttagatccttaagctcgacacataagaccgattcatgtacttttcatccttaaaagatagatgtatatgctacagaaaatggtgatgctggaatgaatggaagctttcttgggaaccaagagataggatggccaagttcaagaacattggatacaagagtgatgaggcggccagtgtcgtcaccgtcatggcagatcaatccaatgaatgtatttagtcaaggttcagttggtggaggagggacaagcttctcatctccagagattatggacactaaactagagagctacaagggaattggcgactcaaactgcgcattgagcttgttaagcaatccacatcaaccacatgacaacaacaacaacaacaacaacaacaacaacaacaacaacaatacatggcgagcttcttcaggttttggcccgatgacggttacaatggctcaaccaccacctgcacctagccagcatcagtatctgaacccgccttgggtattcaaggacaatgataatgatatgtctcctgttttgaatttaggtcgatacaccgagccagataattgtcagataagtagtggcacggcaatgggtgagttcgagttatctgatcaccatcatcaaagtaggagacagtacatggaagatgagaacacaagggcttatgactcttcttctcaccataccaactggtctctcgctgcggctgctgccgctgcggcagcgatgagcaagggcgaggagctgttcaccggggtggtgcccatcctggtcgagctggacggcgacgtaaacggccacaagttcagcgtgtccggcgagggcgagggcgatgccacctacggcaagctgaccctgaagctgatctgcaccaccggcaagctgcccgtgccctggcccaccctcgtgaccaccctgggctacggcctgcagtgcttcgcccgctaccccgaccacatgaagcagcacgacttcttcaagtccgccatgcccgaaggctacgtccaggagcgcaccatcttcttcaaggacgacggcaactacaagacccgcgccgaggtgaagttcgagggcgacaccctggtgaaccgcatcgagctgaagggcatcgacttcaaggaggacggcaacatcctggggcacaagctggagtacaactacaacagccacaacgtctatatcaccgccgacaagcagaagaacggcatcaaggccaacttcaagatccgccacaacatcgaggacggcggcgtgcagctcgccgaccactaccagcagaacacccccatcggcgacggccccgtgctgctgcccgacaaccactacctgagctaccagtccgccctgagcaaagaccccaacgagaagcgcgatcacatggtcctgctggagttcgtgaccgccgccgggatcactctcggcatggacgagctgtacaagtaa

SEQ ID NO: 16 - DNA, 58 bp, synthetic construct
  source 1..58: mol_type = other DNA; note = rSPL9
tacaagggaattggcgactcaaactgcgcattgagcttgttaagcaatccacatcaac

SEQ ID NO: 17 - DNA, 58 bp, Arabidopsis thaliana
  source 1..58: mol_type = genomic DNA; note = A. thaliana SPL9 (AtSPL9)
tacaagggaattggcgactcaaactgtgctctctctcttctgtcaaatccacatcaac